European Patent Specification EP 3 984 642 B1, published September 6, 2023. Title: METHODS AND SYSTEMS FOR NUCLEIC ACID ANALYSIS AND QUANTIFICATION. Applicant: Combinati Incorporated. Application EP 17 871760.9. The sequence listing filed with the application follows.

SEQUENCE LISTING (3 sequences)

SEQ ID NO: 1 - DNA, 22 bp, Artificial Sequence
  Description of Artificial Sequence: Synthetic primer
gcctcaataaagcttgccttga

SEQ ID NO: 2 - DNA, 18 bp, Artificial Sequence
  Description of Artificial Sequence: Synthetic primer
ggggcgcactgctagaga

SEQ ID NO: 3 - DNA, 26 bp, Artificial Sequence
  Description of Artificial Sequence: Synthetic probe
ccagagtcacacaacagacgggcaca